European Patent Application EP 4 321 869 A1, published February 14, 2024. Title: A biomarker for neurodegenerative diseases containing a glycotoxin, a specific protein bound to glycotoxin, or glycotoxin-specific protein complex. Applicant: Gachon University of Industry-Academic cooperation Foundation Veterans Health Service Medical Center. The sequence listing filed with the application follows.

SEQUENCE LISTING (16 sequences)

SEQ ID NO: 1 - DNA, 22 bp, Artificial Sequence
  Col1a1_forward
cctcagggtattgctggacaac

SEQ ID NO: 2 - DNA, 22 bp, Artificial Sequence
  Col1a1_reverse
cagaaggaccttgtttgccagg

SEQ ID NO: 3 - DNA, 22 bp, Artificial Sequence
  Col2a1_forward
gctggtgaagaaggcaaacgag

SEQ ID NO: 4 - DNA, 22 bp, Artificial Sequence
  Col2a1_reverse
ccatcttgacctgggaatccac

SEQ ID NO: 5 - DNA, 23 bp, Artificial Sequence
  Col3a1_forward
gaccaaaaggtgatgctggacag

SEQ ID NO: 6 - DNA, 22 bp, Artificial Sequence
  Col3a1_reverse
caagacctcgtgctccagttag

SEQ ID NO: 7 - DNA, 22 bp, Artificial Sequence
  Col4a1_forward
atggcttgcctggagagatagg

SEQ ID NO: 8 - DNA, 22 bp, Artificial Sequence
  Col4a1_reverse
tggttgccctttgagtcctgga

SEQ ID NO: 9 - DNA, 17 bp, Artificial Sequence
  Col5a1_forward
ggactcggcggaacatt

SEQ ID NO: 10 - DNA, 21 bp, Artificial Sequence
  Col5a1_reverse
ggagttgagggaaccaaagat

SEQ ID NO: 11 - DNA, 22 bp, Artificial Sequence
  Col6a1_forward
gacacctctcagtgtgctctgt

SEQ ID NO: 12 - DNA, 23 bp, Artificial Sequence
  Col6a1_reverse
gcgataagccttggcaggaaatg

SEQ ID NO: 13 - DNA, 21 bp, Artificial Sequence
  Col17a1_forward
gaaaggagacaaaggtgacca

SEQ ID NO: 14 - DNA, 20 bp, Artificial Sequence
  Col17a1_reverse
cggcttgatggcaatacttc

SEQ ID NO: 15 - DNA, 18 bp, Artificial Sequence
  Gapdh_forward
ccatggagaaggctgggg

SEQ ID NO: 16 - DNA, 20 bp, Artificial Sequence
  Gapdh_reverse
caaagttgtcatggatgacc